European Patent Specification EP 3 520 809 B1, published August 6, 2025. Title: IMMUNOSTIMULATORY COMPOSITIONS, PARTICLES, AND USES RELATED THERETO. Applicant: EMORY UNIVERSITY Selvaraj, Periasamy. The sequence listing filed with the application follows.

SEQUENCE LISTING (8 sequences)

SEQ ID NO: 1 - protein, 288 aa, Homo sapiens
MGHTRRQGTSPSKCPYLNFFQLLVLAGLSHFCSGVIHVTKEVKEVATLSCGHNVSVEELAQTRIYWQKEKKMVLTMMSGDMNIWPEYKNRTIFDITNNLSIVILALRPSDEGTYECVVLKYEKDAFKREHLAEVTLSVKADFPTPSISDFEIPTSNIRRIICSTSGGFPEPHLSWLENGEELNAINTTVSQDPETELYAVSSKLDFNMTTNHSFMCLIKYGHLRVNQTFNWNTTKQEHFPDNLLPSWAITLISVNGIFVICCLTYCFAPRCRERRRNERLRRESVRPV

SEQ ID NO: 2 - protein, 208 aa, Homo sapiens [sequence omitted]

SEQ ID NO: 3 - protein, 126 aa, Homo sapiens
KAMHVAQPAVVLASSRGIASFVCEYASPGKATEVRVTVLRQADSQVTEVCAATYMMGNELTFLDDSICTGTSSGNQVNLTIQGLRAMDTGLYICKVELMYPPPYYLGIGNGAQIYVIDPEPCPDSD

SEQ ID NO: 4 - protein, 607 aa, Homo sapiens
TQVCTGTDMKLRLPASPETHLDMLRHLYQGCQVVQGNLELTYLPTNASLSFLQDIQEVQGYVLIAHNQVRQVPLQRLRIVRGTQLFEDNYALAVLDNGDPLNNTTPVTGASPGGLRELQLRSLTEILKGGVLIQRNPQLCYQDTILWKDIFHKNNQLALTLIDTNRSRACHPCSPMCKGSRCWGESSEDCQSLTRTVCAGGCARCKGPLPTDCCHEQCAAGCTGPKHSDCLACLHFNHSGICELHCPALVTYNTDTFESMPNPEGRYTFGASCVTACPYNYLSTDVGSCTLVCPLHNQEVTAEDGTQRCEKCSKPCARVCYGLGMEHLREVRAVTSANIQEFAGCKKIFGSLAFLPESFDGDPASNTAPLQPEQLQVFETLEEITGYLYISAWPDSLPDLSVFQNLQVIRGRILHNGAYSLTLQGLGISWLGLRSLRELGSGLALIHHNTHLCFVHTVPWDQLFRNPHQALLHTANRPEDECVGEGLACHQLCARGHCWGPGPTQCVNCSQFLRGQECVEECRVLQGLPREYVNARHCLPCHPECQPQNGSVTCFGPEADQCVACAHYKDPPFCVARCPSGVKPDLSYMPIWKFPDEEGACQPCPIN

SEQ ID NO: 5 - protein, 214 aa, Homo sapiens
DIQMTQSPSSLSASVGDRVTITCRASQDVNTAVAWYQQKPGKAPKLLIYSASFLYSGVPSRFSGSRSGTDFTLTISSLQPEDFATYYCQQHYTTPPTFGQGTKVEIKRTVAAPSVFIFPPSDEQLKSGTASVVCLLNNFYPREAKVQWKVDNALQSGNSQESVTEQDSKDSTYSLSSTLTLSKADYEKHKVYACEVTHQGLSSPVTKSFNRGEC

SEQ ID NO: 6 - protein, 55 aa, Homo sapiens
GTSHLVKCAEKEKTFCVNGGECFMVKDLSNPSRYLCKCPNEFTGDRCQNYVMASF

SEQ ID NO: 7 - protein, 2254 aa, Homo sapiens
AAGGGGAGGTAACCCTGGCCCCTTTGGTCGGGGCCCCGGGCAGCCGCGCGCCCCTTCCCACGGGGCCCTTTACTGCGCCGCGCGCCCGGCCCCCACCCCTCGCAGCACCCCGCGCCCCGCGCCCTCCCAGCCGGGTCCAGCCGGAGCCATGGGGCCGGAGGATATCCCGCAGTGAGCACCATGGAGCTGGCGGCCTTGTGCCGCTGGGGGCTCCTCCTCGCCCTCTTGCCCCCCGGAGCCGCGAGCACCCAAGTGTGCACCGGCACAGACATGAAGCTGCGGCTCCCTGCCAGTCCCGAGACCCACCTGGACATGCTCCGCCACCTCTACCAGGGCTGCCAGGTGGTGCAGGGAAACCTGGAACTCACCTACCTGCCCACCAATGCCAGCCTGTCCTTCCTGCAGGATATCCAGGAGGTGCAGGGCTACGTGCTCATCGCTCACAACCAAGTGAGGCAGGTCCCACTGCAGAGGCTGCGGATTGTGCGAGGCACCCAGCTCTTTGAGGACAACTATGCCCTGGCCGTGCTAGACAATGGAGACCCGCTGAACAATACCACCCCTGTCACAGGGGCCTCCCCAGGAGGCCTGCGGGAGCTGCAGCTTCGAAGCCTCACAGAGATCTTGAAAGGAGGGGTCTTGATCCAGCGGAACCCCCAGCTCTGCTACCAGGACACGATTTTGTGGAAGGACATCTTCCACAAGAACAACCAGCTGGCTCTCACACTGATAGACACCAACCGCTCTCGGGCCTGCCACCCCTGTTCTCCGATGTGTAAGGGCTCCCGCTGCTGGGGAGAGAGTTCTGAGGATTGTCAGAGCCTGACGCGCACTGTCTGTGCCGGTGGCTGTGCCCGCTGCAAGGGGCCACTGCCCACTGACTGCTGCCATGAGCAGTGTGCTGCCGGCTGCACGGGCCCCAAGCACTCTGACTGCCTGGCCTGCCTCCACTTCAACCACAGTGGCATCTGTGAGCTGCACTGCCCAGCCCTGGTCACCTACAACACAGACACGTTTGAGTCCATGCCCAATCCCGAGGGCCGGTATACATTCGGCGCCAGCTGTGTGACTGCCTGTCCCTACAACTACCTTTCTACGGACGTGGGATCCTGCACCCTCGTCTGCCCCCTGCACAACCAAGAGGTGACAGCAGAGGATGGAACACAGCGGTGTGAGAAGTGCAGCAAGCCCTGTGCCCGAGTGTGCTATGGTCTGGGCATGGAGCACTTGCGAGAGGTGAGGGCAGTTACCAGTGCCAATATCCAGGAGTTTGCTGGCTGCAAGAAGATCTTTGGGAGCCTGGCATTTCTGCCGGAGAGCTTTGATGGGGACCCAGCCTCCAACACTGCCCCGCTCCAGCCAGAGCAGCTCCAAGTGTTTGAGACTCTGGAAGAGATCACAGGTTACCTATACATCTCAGCATGGCCGGACAGCCTGCCTGACCTCAGCGTCTTCCAGAACCTGCAAGTAATCCGGGGACGAATTCTGCACAATGGCGCCTACTCGCTGACCCTGCAAGGGCTGGGCATCAGCTGGCTGGGGCTGCGCTCACTGAGGGAACTGGGCAGTGGACTGGCCCTCATCCACCATAACACCCACCTCTGCTTCGTGCACACGGTGCCCTGGGACCAGCTCTTTCGGAACCCGCACCAAGCTCTGCTCCACACTGCCAACCGGCCAGAGGACGAGTGTGTGGGCGAGGGCCTGGCCTGCCACCAGCTGTGCGCCCGAGGGCACTGCTGGGGTCCAGGGCCCACCCAGTGTGTCAACTGCAGCCAGTTCCTTCGGGGCCAGGAGTGCGTGGAGGAATGCCGAGTACTGCAGGGGCTCCCCAGGGAGTATGTGAATGCCAGGCACTGTTTGCCGTGCCACCCTGAGTGTCAGCCCCAGAATGGCTCAGTGACCTGTTTTGGACCGGAGGCTGACCAGTGTGTGGCCTGTGCCCACTATAAGGACCCTCCCTTCTGCGTGGCCCGCTGCCCCAGCGGTGTGAAACCTGACCTCTCCTACATGCCCATCTGGAAGTTTCCAGATGAGGAGGGCGCATGCCAGCCTTGCCCCATCAACTGCACCCACTCCTGTGTGGACCTGGATGACAAGGGCTGCCCCGCCGAGCAGAGAGCCAGCCCTCTGACGGAATTCCTTGAAAATGGTGGGACATCCTTATCAGAGAAAACAGTTCTTCTGCTGGTGACTCCATTTCTGGCAGCAGCCTGGAGCCTTCATCCCTAACAGAAGGCCAAGGGGCCCTCCG

SEQ ID NO: 8 - protein, 22 aa, Homo sapiens
TGACTGTGAACGTTCGAGATGA